European Patent Application EP 4 613 259 A1, published September 10, 2025. Title: PHARMACEUTICAL, DERMATOLOGICAL OR COSMETIC COMPOUNDS AND COMPOSITIONS FOR REDUCING MELANIN SYNTHESIS, STIMULATING TYPE I COLLAGEN PRODUCTION, DEPIGMENTING THE SKIN AND/OR PROMOTING AN ANTI-AGING ACTION OF THE SKIN IN AN INDIVIDUAL OR ANIMAL, USES AND METHODS. Applicant: Chemyunion Ltda. Application WO PCTBR2023050367, filed October 30, 2023. The sequence listing filed with the application follows.

SEQUENCE LISTING (5 sequences)

SEQ ID NO: 1 - protein, 4 aa, synthetic construct
  BINDING 1: note = N-palmitoylated
QHWV

SEQ ID NO: 2 - protein, 4 aa, synthetic construct
  BINDING 1: note = N-acetylated
QHWV

SEQ ID NO: 3 - protein, 4 aa, synthetic construct
  BINDING 1: note = N-acetylated
QHYV

SEQ ID NO: 4 - protein, 4 aa, synthetic construct
  BINDING 1: note = N-palmitoylated
SHWV

SEQ ID NO: 5 - protein, 4 aa, synthetic construct
  BINDING 1: note = N-palmitoylated
QHYV